European Patent Application EP 4 342 467 A1, published March 27, 2024. Title: Ku inhibitors for use in tumor therapy. Applicant: Masarykova univerzita. Application EP. The sequence listing filed with the application follows.

SEQUENCE LISTING (6 sequences)

SEQ ID NO: 1 - DNA, 25 bp, synthetic construct
  source 1..25: mol_type = other DNA
cacaacgaccacctagatggatcca

SEQ ID NO: 2 - DNA, 25 bp, synthetic construct
  source 1..25: mol_type = other DNA
tggatccatctaggtggtcgttgtg

SEQ ID NO: 3 - DNA, 22 bp, synthetic construct
  source 1..22: mol_type = other DNA
atgaaagctgggtttgcttttg

SEQ ID NO: 4 - DNA, 18 bp, synthetic construct
  source 1..18: mol_type = other DNA
cgtcccttacgcccaaat

SEQ ID NO: 5 - DNA, 98 bp, Arabidopsis thaliana
  source 1..98: mol_type = other DNA
atgaaagctgggtttgcttttgtatacatggaagatgaaagggatgcggaagatgccatccgagcacttgaccgctttgaatttgggcgtaagggacg

SEQ ID NO: 6 - DNA, 24 bp, synthetic construct
  source 1..24: mol_type = other DNA
ccctaaccctaaccctaaccctaa